European Patent Specification EP 3 049 525 B1, published July 23, 2025. Title: INTERLEUKIN-4 RECEPTOR-BINDING FUSION PROTEINS AND USES THEREOF. Applicant: MEDICENNA THERAPEUTICS PTE LTD MERCHANT, Fahar. The sequence listing filed with the application follows.

SEQUENCE LISTING (31 sequences)

SEQ ID NO: 1 - protein, 130 aa, Artificial Sequence
  IL-4 sequence including an additional methionine at the N-terminus
MHKCDITLQEIIKTLNSLTEQKTLCTELTVTDIFAASKNTTEKETFCRAATVLRQFYSHHEKDTRCLGATAQQFHRHKQLIRFLKRLDRNLWGLAGLNSCPVKEANQSTLENFLERLKTIMREKYSKCSS

SEQ ID NO: 2 - protein, 130 aa, Artificial Sequence
  IL-4 sequence including an additional methionine at the N-terminus
MHKCDITLQEIIKTLNSLTEQKTLCTELTVTDIFAASKDTTEKETFCRAATVLRQFYSHHEKDTRCLGATAQQFHRHKQLIRFLKRLDRNLWGLAGLNSCPVKEANQSTLENFLERLKTIMREKYSKCSS

SEQ ID NO: 3 - protein, 134 aa, Artificial Sequence
  circularly permuted IL-4 sequence
MDTTEKETFCRAATVLRQFYSHHEKDTRCLGATAQQFHRHKQLIRFLKRLDRNLWGLAGLNSCPVKEANQSTLENFLERLKTIMREKYSKCSSGGNGGHKCDITLQEIIKTLNSLTEQKTLCTELTVTDIFAAS

SEQ ID NO: 4 - protein, 134 aa, Artificial Sequence
  circularly permuted "RGA" variant IL-4
MDTTEKETFCRAATVLRQFYSHHEKDTRCLGATAQQFHRHKQLIRFLKRLDRNLWGLAGLNSCPVKEANQSTLENFLERLRVIMQSKWFKCGAGGNGGHKCDITLQEIIKTLNSLTEQKTLCTELTVTDIFAAS

SEQ ID NO: 5 - protein, 134 aa, Artificial Sequence
  circularly permuted "KFR" variant IL-4
MDTTEKETFCRAATVLRQFYSHHEKDTRCLGATAQQFHRHKQLIRFLKRLDRNLWGLAGLNSCPVKEANQSTLENFLERLKTIMKEKFRKCSSGGNGGHKCDITLQEIIKTLNSLTEQKTLCTELTVTDIFAAS

SEQ ID NO: 6 - protein, 133 aa, Artificial Sequence
  circularly permuted "KF" variant IL-4
MDTTEKETFCRAATVLRQFYSHHEKDTRCLGATAQQFHRHKQLIRFLKRLDRNLWGLAGLNSCPVKEANQSTLENFLERLKTIMKEKFKCSSGGNGGHKCDITLQEIIKTLNSLTEQKTLCTELTVTDIFAAS

SEQ ID NO: 7 - protein, 114 aa, Artificial Sequence
  IL-13 including an additional methionine at the N-terminus
MPGPVPPSTALRELIEELVNITQNQKAPLCNGSMVWSINLTAGMYCAALESLINVSGCSAIEKTQRMLSGFCPHKVSAGQFSSLHVRDTKIEVAQFVKDLLLHLKKLFREGQFN

SEQ ID NO: 8 - protein, 114 aa, Artificial Sequence
  " A11" IL-13 variant
MPGPVPPSTAVRELIEELINITQNQKAPLCNGSMVWSINRTAGMYCAALESLINVSGCSAIEKTQRMLSGFCPHKVSAGQFSSLHVRSSKIEVAQFVKDLLFHLRTLFREGQFN

SEQ ID NO: 9 - protein, 114 aa, Artificial Sequence
  "DN" IL-13 variant
MPGPVPPSTAVRALIEELINITQNQKAPLCNGSMVWSINLTAGMYCAALESLINVSGCSAIEKTQDMLSGFCPHKVSAGQFSSLHVRSSKIEVAQFVKDLLFHLRTLFREGQFN

SEQ ID NO: 10 - protein, 117 aa, Artificial Sequence
  circularly permuted IL-13
MYCAALESLINVSGCSAIEKTQRMLSGFCPHKVSAGQFSSLHVRDTKIEVAQFVKDLLLHLKKLFREGQFNGGSGPGPVPPSTALRELIEELVNITQNQKAPLCNGSMVWSINLTAG

SEQ ID NO: 11 - protein, 118 aa, Artificial Sequence
  circularly permuted IL-13
MYCAALESLINVSGCSAIEKTQRMLSGFCPHKVSAGQFSSLHVRDTKIEVAQFVKDLLLHLKKLFREGQFNGGSGMPGPVPPSTALRELIEELVNITQNQKAPLCNGSMVWSINLTAG

SEQ ID NO: 12 - protein, 117 aa, Artificial Sequence
  circularly permuted IL-13 "A11" variant
MYCAALESLINVSGCSAIEKTQRMLSGFCPHKVSAGQFSSLHVRSSKIEVAQFVKDLLFHLRTLFREGQFNGGSGPGPVPPSTAVRELIEELINITQNQKAPLCNGSMVWSINRTAG

SEQ ID NO: 13 - protein, 118 aa, Artificial Sequence
  circularly permuted IL-13
MYCAALESLINVSGCSAIEKTQRMLSGFCPHKVSAGQFSSLHVRSSKIEVAQFVKDLLFHLRTLFREGQFNGGSGMPGPVPPSTAVRELIEELINITQNQKAPLCNGSMVWSINRTAG

SEQ ID NO: 14 - protein, 117 aa, Artificial Sequence
  circularly permuted "DN" IL-13
MYCAALESLINVSGCSAIEKTQDMLSGFCPHKVSAGQFSSLHVRSSKIEVAQFVKDLLFHLRTLFREGQFNGGSGPGPVPPSTAVRALIEELINITQNQKAPLCNGSMVWSINLTAG

SEQ ID NO: 15 - protein, 118 aa, Artificial Sequence
  circularly permuted IL-13
MYCAALESLINVSGCSAIEKTQDMLSGFCPHKVSAGQFSSLHVRSSKIEVAQFVKDLLFHLRTLFREGQFNGGSGMPGPVPPSTAVRALIEELINITQNQKAPLCNGSMVWSINLTAG

SEQ ID NO: 16 - protein, 232 aa, Homom sapiens
SQSNRELVVDFLSYKLSQKGYSWSQFSDVEENRTEAPEGTESEMETPSAINGNPSWHLADSPAVNGATGHSSSLDAREVIPMAAVKQALREAGDEFELRYRRAFSDLTSQLHITPGTAYQSFEQVVNELFRDGVNWGRIVAFFSFGGALCVESVDKEMQVLVSRIAAWMATYLNDHLEPWIQENGGWDTFVELYGNNAAAESRKGQERFNRWFLTGMTVAGVVLLGSLFSRK

SEQ ID NO: 17 - protein, 7 aa, Artificial Sequence
  linker
KASGGPE

SEQ ID NO: 18 - protein, 373 aa, Artificial Sequence
  cpIL-4-BclxL
MDTTEKETFCRAATVLRQFYSHHEKDTRCLGATAQQFHRHKQLIRFLKRLDRNLWGLAGLNSCPVKEANQSTLENFLERLKTIMREKYSKCSSGGNGGHKCDITLQEIIKTLNSLTEQKTLCTELTVTDIFAASKASGGPESQSNRELVVDFLSYKLSQKGYSWSQFSDVEENRTEAPEGTESEMETPSAINGNPSWHLADSPAVNGATGHSSSLDAREVIPMAAVKQALREAGDEFELRYRRAFSDLTSQLHITPGTAYQSFEQVVNELFRDGVNWGRIVAFFSFGGALCVESVDKEMQVLVSRIAAWMATYLNDHLEPWIQENGGWDTFVELYGNNAAAESRKGQERFNRWFLTGMTVAGVVLLGSLFSRK

SEQ ID NO: 19 - protein, 82 aa, Artificial Sequence
  ubiquitin linker
GGGSMQIFVRTLTGRTITLEVEPSDTIENVRARIQDREGIPPDQQRLIFAGRQLEDGRTLSDYNIQRESTLHLVLRLRGGGS

SEQ ID NO: 20 - protein, 448 aa, Artificial Sequence
  cpIL-4-Ub-BclxL
MDTTEKETFCRAATVLRQFYSHHEKDTRCLGATAQQFHRHKQLIRFLKRLDRNLWGLAGLNSCPVKEANQSTLENFLERLKTIMREKYSKCSSGGNGGHKCDITLQEIIKTLNSLTEQKTLCTELTVTDIFAASGGGSMQIFVRTLTGRTITLEVEPSDTIENVRARIQDREGIPPDQQRLIFAGRQLEDGRTLSDYNIQRESTLHLVLRLRGGGSSQSNRELVVDFLSYKLSQKGYSWSQFSDVEENRTEAPEGTESEMETPSAINGNPSWHLADSPAVNGATGHSSSLDAREVIPMAAVKQALREAGDEFELRYRRAFSDLTSQLHITPGTAYQSFEQVVNELFRDGVNWGRIVAFFSFGGALCVESVDKEMQVLVSRIAAWMATYLNDHLEPWIQENGGWDTFVELYGNNAAAESRKGQERFNRWFLTGMTVAGVVLLGSLFSRK

SEQ ID NO: 21 - protein, 448 aa, Artificial Sequence
  cpKRF4-Ub-BclxL
MDTTEKETFCRAATVLRQFYSHHEKDTRCLGATAQQFHRHKQLIRFLKRLDRNLWGLAGLNSCPVKEANQSTLENFLERLKTIMKEKFRKCSSGGNGGHKCDITLQEIIKTLNSLTEQKTLCTELTVTDIFAASGGGSMQIFVRTLTGRTITLEVEPSDTIENVRARIQDREGIPPDQQRLIFAGRQLEDGRTLSDYNIQRESTLHLVLRLRGGGSSQSNRELVVDFLSYKLSQKGYSWSQFSDVEENRTEAPEGTESEMETPSAINGNPSWHLADSPAVNGATGHSSSLDAREVIPMAAVKQALREAGDEFELRYRRAFSDLTSQLHITPGTAYQSFEQVVNELFRDGVNWGRIVAFFSFGGALCVESVDKEMQVLVSRIAAWMATYLNDHLEPWIQENGGWDTFVELYGNNAAAESRKGQERFNRWFLTGMTVAGVVLLGSLFSRK

SEQ ID NO: 22 - protein, 369 aa, Artificial Sequence
  cpKFR4-BclxL
MDTTEKETFCRAATVLRQFYSHHEKDTRCLGATAQQFHRHKQLIRFLKRLDRNLWGLAGLNSCPVKEANQSTLENFLERLKTIMKEKFRKCSSGGNGGHKCDITLQEIIKTLNSLTEQKTLCTELTVTDIFAASKGSSQSNRELVVDFLSYKLSQKGYSWSQFSDVEENRTEAPEGTESEMETPSAINGNPSWHLADSPAVNGATGHSSSLDAREVIPMAAVKQALREAGDEFELRYRRAFSDLTSQLHITPGTAYQSFEQVVNELFRDGVNWGRIVAFFSFGGALCVESVDKEMQVLVSRIAAWMATYLNDHLEPWIQENGGWDTFVELYGNNAAAESRKGQERFNRWFLTGMTVAGVVLLGSLFSRK

SEQ ID NO: 23 - protein, 449 aa, Artificial Sequence
  cpS4-Ub-BclxL
MDTTEKETFCRAATVLRQFYSHHEKDTRCLGATAQQFHRHKQLIRFLKRLDRNLWGLAGLNSCPVKEANQSTLENFLERLRVIMQSKWFKCGAGGNGGHKCDITLQEIIKTLNSLTEQKTLCTELTVTDIFAASKGGGSMQIFVRTLTGRTITLEVEPSDTIENVRARIQDREGIPPDQQRLIFAGRQLEDGRTLSDYNIQRESTLHLVLRLRGGGSSQSNRELVVDFLSYKLSQKGYSWSQFSDVEENRTEAPEGTESEMETPSAINGNPSWHLADSPAVNGATGHSSSLDAREVIPMAAVKQALREAGDEFELRYRRAFSDLTSQLHITPGTAYQSFEQVVNELFRDGVNWGRIVAFFSFGGALCVESVDKEMQVLVSRIAAWMATYLNDHLEPWIQENGGWDTFVELYGNNAAAESRKGQERFNRWFLTGMTVAGVVLLGSLFSRK

SEQ ID NO: 24 - protein, 369 aa, Artificial Sequence
  cpS4-BclxL
MDTTEKETFCRAATVLRQFYSHHEKDTRCLGATAQQFHRHKQLIRFLKRLDRNLWGLAGLNSCPVKEANQSTLENFLERLRVIMQSKWFKCGAGGNGGHKCDITLQEIIKTLNSLTEQKTLCTELTVTDIFAASKGSSQSNRELVVDFLSYKLSQKGYSWSQFSDVEENRTEAPEGTESEMETPSAINGNPSWHLADSPAVNGATGHSSSLDAREVIPMAAVKQALREAGDEFELRYRRAFSDLTSQLHITPGTAYQSFEQVVNELFRDGVNWGRIVAFFSFGGALCVESVDKEMQVLVSRIAAWMATYLNDHLEPWIQENGGWDTFVELYGNNAAAESRKGQERFNRWFLTGMTVAGVVLLGSLFSRK

SEQ ID NO: 25 - DNA, 390 bp, Artificial Sequence
  IL-4
atgcacaaatgcgacattaccctgcaagagatcattaagaccctgaacagcctgaccgagcaaaagaccctgtgtaccgaactgaccgtcacggacatcttcgctgcgtccaaggacactacggaaaaggaaacgttctgtcgtgcggcgacggtgctgcgccagttctacagccaccatgagaaagatacccgttgcctcggtgcgaccgcgcaacagttccaccgtcacaaacagctgattcgcttcctgaagcgtctggatcgcaacctgtggggtttggcgggtctgaactcctgtccagtcaaagaagccaatcagtctacgctggaaaactttttggagcgtctgaaaactatcatgcgtgagaagtacagcaaatgcagcagc

SEQ ID NO: 26 - DNA, 402 bp, Artificial Sequence
  cpIL4
atggataccaccgagaaagaaacgttctgccgtgctgccactgtcctgcgccagttttacagccatcacgaaaaggacacccgttgcctgggtgcgacggcgcagcaattccaccgccacaaacagctgattcgtttcctgaagcgtctggaccgtaacctgtggggtctggcgggtctgaacagctgtccagtgaaagaagcgaatcagagcaccttggagaatttcctcgaacgcctgaaaaccatcatgcgtgagaaatacagcaagtgttctagcggcggtaacggtggccacaaatgcgatatcaccctgcaagagatcattaagacgctgaactccttgacggaacaaaagaccctgtgtactgagctgacggtcaccgacattttcgcggcgtcc

SEQ ID NO: 27 - DNA, 402 bp, Artificial Sequence
  cpKFR
atggatactaccgagaaagaaacgttttgccgtgctgcgaccgtcctgcgtcagttctacagccaccacgaaaaggacacccgctgtctgggtgcgactgcccaacaattccatcgtcacaaacagctgattcgtttcctgaagcgtctggaccgcaacctgtggggtctggcgggcttgaactcctgcccagtcaaagaagcgaaccaaagcaccctggaaaacttcttggagcgtctgaaaacgatcatgaaagagaagttccgcaagtgtagcagcggtggtaatggtggccacaagtgcgacattacgctgcaggaaatcattaagaccctgaactctctgaccgagcagaaaaccctctgtaccgagctgacggtgacggatatctttgcggcgagc

SEQ ID NO: 28 - DNA, 402 bp, Artificial Sequence
  cpS4
atggataccaccgaaaaagaaactttttgtcgtgccgcgactgtcctgcgccagttctacagccaccacgaaaaggacacccgttgcctgggtgcgaccgctcaacaattccatcgccacaaacagctgattcgtttcctgaaacgtctggatcgcaacctgtggggtctggcgggtttgaacagctgtccagtcaaagaagcgaaccagagcaccctggaaaactttctggagcgtctgcgtgttatcatgcagagcaagtggttcaagtgcggtgcgggtggcaatggtggccacaagtgtgacattaccttgcaagagattatcaaaacgctgaactctctgaccgagcaaaagacgctgtgcaccgagctgacggtgacggacatcttcgcggcgtcc

SEQ ID NO: 29 - DNA, 696 bp, Artificial Sequence
  variant BclxL
tctcagtctaaccgcgaactggtggtggacttcctgtcttataaactgagccagaaaggctactcctggagccagttcagcgacgtagaggagaaccgtaccgaagctcctgaaggcaccgagagcgagatggaaaccccatccgcgattaacggcaacccgtcctggcacctggctgattctccggcggtaaacggcgcaactggtcattctagctccctggatgcacgtgaagtaatcccgatggccgcggttaaacaggcgctgcgtgaagctggtgacgaatttgagctgcgctaccgccgtgcattttctgatctgacctcccagctgcacatcacgccgggtaccgcataccaaagcttcgaacaggtggttaacgaactgtttcgtgacggcgtcaactggggccgcatcgtggcctttttctctttcggcggtgccctgtgcgtcgaatctgttgacaaagaaatgcaggttctggtgagccgtattgcggcttggatggcaacttatctgaacgatcacctggaaccgtggatccaggaaaacggtggttgggataccttcgttgaactgtacggtaacaatgctgcggcggaatcccgtaagggtcaagaacgtttcaatcgctggttcctgaccggcatgactgttgctggtgtagttctgctgggttctctgttctcccgtaaa

SEQ ID NO: 30 - DNA, 1119 bp, Artificial Sequence
  cpIL4-BclxL
atggacacgactgagaaagagaccttctgccgtgcagcaactgttctgcgtcagttctattcccaccacgaaaaagatacgcgttgcctgggtgctactgcgcagcagttccatcgtcataagcaactgattcgctttctgaaacgtctggaccgtaacctgtggggtctggccggtctgaacagctgcccggtcaaagaagcgaaccagtccactctggaaaacttcctggaacgcctgaagaccatcatgcgcgaaaaatactccaagtgttccagcggcggcaacggcggtcacaaatgtgacatcaccctgcaggaaatcatcaaaactctgaattctctgactgagcagaaaaccctgtgtaccgaactgaccgtgaccgatatttttgccgcttctaaagcgtctggtggcccggaatctcagtctaaccgcgaactggtggtggacttcctgtcttataaactgagccagaaaggctactcctggagccagttcagcgacgtagaggagaaccgtaccgaagctcctgaaggcaccgagagcgagatggaaaccccatccgcgattaacggcaacccgtcctggcacctggctgattctccggcggtaaacggcgcaactggtcattctagctccctggatgcacgtgaagtaatcccgatggccgcggttaaacaggcgctgcgtgaagctggtgacgaatttgagctgcgctaccgccgtgcattttctgatctgacctcccagctgcacatcacgccgggtaccgcataccaaagcttcgaacaggtggttaacgaactgtttcgtgacggcgtcaactggggccgcatcgtggcctttttctctttcggcggtgccctgtgcgtcgaatctgttgacaaagaaatgcaggttctggtgagccgtattgcggcttggatggcaacttatctgaacgatcacctggaaccgtggatccaggaaaacggtggttgggataccttcgttgaactgtacggtaacaatgctgcggcggaatcccgtaagggtcaagaacgtttcaatcgctggttcctgaccggcatgactgttgctggtgtagttctgctgggttctctgttctcccgtaaa

SEQ ID NO: 31 - DNA, 1347 bp, Artificial Sequence
  cpIL4-Ub-BclxL
atggacacgactgagaaagagaccttctgccgtgcagcaactgttctgcgtcagttctattcccaccacgaaaaagatacgcgttgcctgggtgctactgcgcagcagttccatcgtcataagcaactgattcgctttctgaaacgtctggaccgtaacctgtggggtctggccggtctgaacagctgcccggtcaaagaagcgaaccagtccactctggaaaacttcctggaacgcctgaagaccatcatgcgcgaaaaatactccaagtgttccagcggcggcaacggcggtcacaaatgtgacatcaccctgcaggaaatcatcaaaactctgaattctctgactgagcagaaaaccctgtgtaccgaactgaccgtgaccgatatttttgccgcttctaaaggtggcggctctatgcaaattttcgttcgtaccctgacgggtcgtaccatcactctggaagtagaaccgagcgacacgatcgaaaatgtccgcgcacgcatccaagaccgcgaaggcattccaccggatcagcagcgtctgatcttcgccggtcgccagctggaggatggtcgtactctgtccgattataacatccagcgtgaatccaccctgcacctggtgctgcgtctgcgtggcggtggtagctctcagtctaaccgcgaactggtggtggacttcctgtcttataaactgagccagaaaggctactcctggagccagttcagcgacgtagaggagaaccgtaccgaagctcctgaaggcaccgagagcgagatggaaaccccatccgcgattaacggcaacccgtcctggcacctggctgattctccggcggtaaacggcgcaactggtcattctagctccctggatgcacgtgaagtaatcccgatggccgcggttaaacaggcgctgcgtgaagctggtgacgaatttgagctgcgctaccgccgtgcattttctgatctgacctcccagctgcacatcacgccgggtaccgcataccaaagcttcgaacaggtggttaacgaactgtttcgtgacggcgtcaactggggccgcatcgtggcctttttctctttcggcggtgccctgtgcgtcgaatctgttgacaaagaaatgcaggttctggtgagccgtattgcggcttggatggcaacttatctgaacgatcacctggaaccgtggatccaggaaaacggtggttgggataccttcgttgaactgtacggtaacaatgctgcggcggaatcccgtaagggtcaagaacgtttcaatcgctggttcctgaccggcatgactgttgctggtgtagttctgctgggttctctgttctcccgtaaa